European Patent Application EP 4 534 555 A1, published April 9, 2025. Title: PREPARATION METHOD FOR BIOSYNTHETIC HUMAN BODY STRUCTURAL MATERIAL. Applicant: SHANXI JINBO BIO-PHARMACEUTICAL CO., LTD. The sequence listing filed with the application follows.

SEQUENCE LISTING (52 sequences)

SEQ ID NO: 1 - protein, 285 aa, synthetic construct
  REGION 1..285: note = the amino acid sequence of the recombinant type IV humanized collagen C007
GQKGDQGEKGQIGPIGEKGSRGDPGTPGVPGKDGQAGQPGQPGPKGDPGISGTPGAPGLPGPKGSVGGMGLPGTPGEKGVPGIPGPQGSPGLPGDKGAKGEKGQAGPPGIGIPGLRGEKGDQGIAGFPGSPGEKGEKGSIGIPGMPGSPGLKGSPGSVGYPGSPGLPGEKGDKGLPGLDGIPGVKGEAGLPGTPGPTGPAGQKGEPGSDGIPGSAGEKGEPGLPGRGFPGFPGAKGDKGSKGEVGFPGLAGSPGIPGSKGEQGFMGPPGPQGQPGLPGSPGHATE

SEQ ID NO: 2 - protein, 342 aa, synthetic construct
  REGION 1..342: note = the amino acid sequence of the recombinant type IV humanized collagen C4P7C6
GFPGFPGAKGDKGSKGEVGFPGLAGSPGIPGSKGEQGFMGPPGPQGQPGLPGSPGHAGFPGFPGAKGDKGSKGEVGFPGLAGSPGIPGSKGEQGFMGPPGPQGQPGLPGSPGHAGFPGFPGAKGDKGSKGEVGFPGLAGSPGIPGSKGEQGFMGPPGPQGQPGLPGSPGHAGFPGFPGAKGDKGSKGEVGFPGLAGSPGIPGSKGEQGFMGPPGPQGQPGLPGSPGHAGFPGFPGAKGDKGSKGEVGFPGLAGSPGIPGSKGEQGFMGPPGPQGQPGLPGSPGHAGFPGFPGAKGDKGSKGEVGFPGLAGSPGIPGSKGEQGFMGPPGPQGQPGLPGSPGHA

SEQ ID NO: 3 - protein, 308 aa, synthetic construct
  REGION 1..308: note = the amino acid sequence of the recombinant type IV humanized collagen C4P7E5
GLPGTPGPTGPAGQKGEPGSDGIPGSAGEKGEPGLPGRGFPGFPGAKGDKGSKGEVGFPGLAGSPGIPGSKGEQGFMGLPGTPGPTGPAGQKGEPGSDGIPGSAGEKGEPGLPGRGFPGFPGAKGDKGSKGEVGFPGLAGSPGIPGSKGEQGFMGLPGTPGPTGPAGQKGEPGSDGIPGSAGEKGEPGLPGRGFPGFPGAKGDKGSKGEVGFPGLAGSPGIPGSKGEQGFMGLPGTPGPTGPAGQKGEPGSDGIPGSAGEKGEPGLPGRGFPGFPGAKGDKGSKGEVGFPGLAGSPGIPGSKGEQGFM

SEQ ID NO: 4 - DNA, 873 bp, synthetic construct
  misc_feature 1..873: note = the polynucleotide sequence of the recombinant type IV humanized collagen C007
  source 1..873: mol_type = other DNA
gaaaacctgtatttccagggtcagaaaggagatcaaggagaaaaaggacagataggaccaataggagaaaaagggagccggggagatccgggaacaccgggagtgccgggaaaagatggacaggcaggccagccgggacagccgggtcctaaaggagatccgggtataagcggaacaccgggtgcaccgggattacctggtccgaaagggagcgtagggggaatgggactgccgggaacacctggtgaaaaaggcgtacctggtattccgggtcctcaggggtccccgggactgcctggtgataaaggtgcaaaaggggaaaaagggcaagcaggtccgccgggtattggtataccgggtctgcgtggggaaaaaggtgatcagggtattgccggttttccgggtagcccgggtgagaaaggtgaaaaaggaagtataggaataccgggtatgcctggtagtccgggtctgaaaggtagcccgggaagcgtggggtatccgggtagccctggtctgcctggggaaaaaggcgataaaggtctgccgggtctggacggtattcctggtgttaaaggggaagcaggtctgccggggaccccgggtccaacaggtcctgcagggcagaaaggtgaaccaggtagcgatggtattccggggtctgcgggggaaaaaggagaaccgggtctgccgggaagaggttttccgggctttccgggtgcaaaaggagataagggtagcaaaggcgaagtgggttttccgggactggcaggtagtccgggaatccctggtagcaaaggtgaacagggttttatggggccgccgggtccgcagggtcagcctggtttaccgggtagcccaggtcatgcgacagag

SEQ ID NO: 5 - DNA, 1044 bp, synthetic construct
  misc_feature 1..1044: note = the polynucleotide sequence of the recombinant type IV humanized collagen C4P7C6
  source 1..1044: mol_type = other DNA
gaaaatctatatttccaaggatttcccgggttcccgggtgcaaaaggcgacaagggttcgaaaggcgaagttggcttcccgggattagcgggtagcccaggtatcccgggttctaagggtgaacagggtttcatgggtccgcccggcccacagggtcaaccgggcctgcctggtagcccgggtcatgcgggctttccaggtttcccgggcgcgaaaggcgacaaaggtagcaagggcgaagtcggttttccgggccttgctggcagcccgggcatcccggggtccaagggcgagcaaggattcatgggtccgcctggcccacaaggccaaccgggtttgccgggctctccgggtcacgccggttttccgggattcccgggagcgaaaggtgataagggctccaaaggtgaggtgggttttccgggcttggctggcagcccgggtattccgggtagcaagggcgagcagggttttatgggcccgcctggtccgcagggccaaccggggctgccgggctccccgggccacgcaggcttcccaggttttccgggtgcgaaaggcgataaaggtagtaagggtgaagtgggcttcccgggtctcgcgggtagcccgggtattccgggctcgaagggcgaacagggctttatgggcccaccgggtccgcagggtcagccgggcctgccgggtagcccgggccacgcgggtttcccgggcttcccgggtgccaaaggcgataaaggttcaaagggggaggtgggttttccgggtctggcaggcagcccgggcatcccgggcagcaagggcgaacaaggttttatgggtccgcctggaccgcaaggtcagccgggcctgccgggtagtccgggccatgccggcttcccgggttttccgggtgcgaaaggggacaaaggcagcaagggagaggttggtttcccaggcctggctggtagcccgggtattccgggctccaagggtgagcagggtttcatgggtccgcctggcccacagggtcaacctggcctgccgggttctccgggtcatgcg

SEQ ID NO: 6 - DNA, 942 bp, synthetic construct
  misc_feature 1..942: note = the polynucleotide sequence of the recombinant type IV humanized collagen C4P7E5
  source 1..942: mol_type = other DNA
gaaaatttatattttcaagggctacccggaacgccaggtccaactggtccggcgggccaaaaaggcgagccggggtcggacggcatcccgggtagcgcaggcgaaaaaggtgaaccgggcctgccgggccgtggcttcccgggcttcccgggagcgaaaggcgataaaggcagcaagggcgaggtgggttttccgggattggctggtagcccggggattccgggctccaagggcgagcagggttttatgggtctgccgggaaccccaggtccgaccggtccggcgggtcagaaaggtgaaccgggtagcgacggcattccgggcagcgcgggtgaaaaaggtgaaccgggtttgccgggtcgcggttttccgggtttcccgggtgctaaaggcgacaaaggttccaagggtgaagttggttttccgggactggcgggcagcccgggcatcccaggctccaagggcgaacaaggctttatgggtctgccgggcaccccgggtccgaccggtcctgcgggtcaaaagggtgagccgggtagcgatggtattccgggctctgctggcgagaaaggtgagccgggcctgccgggccgtggtttcccgggattccctggtgccaagggtgacaagggttcgaagggcgaggttggttttccgggcctggcgggttctccgggtatcccgggtagcaagggggagcagggttttatgggcttaccgggaaccccgggcccaacgggtccggcaggtcagaaaggggaaccgggcagcgatggtatcccgggcagtgccggtgagaagggcgagccgggcctgcccggccgtggtttccctggtttcccgggtgcaaaaggtgataaaggttccaagggcgaagtgggtttcccgggtctcgcgggcagcccgggcattccggggtctaagggtgagcagggtttcatg

SEQ ID NO: 7 - protein, 6 aa, synthetic construct
  REGION 1..6: note = the amino acid sequence excisable by the TEV protease
ENLYFQ

SEQ ID NO: 8 - protein, 15 aa, synthetic construct
  REGION 1..15: note = Partial sequence of C007 mass spectrometry detection results
GSVGGMGLPGTPGEK

SEQ ID NO: 9 - protein, 18 aa, synthetic construct
  REGION 1..18: note = Partial sequence of C007 mass spectrometry detection results
GVPGIPGPQGSPGLPGDK

SEQ ID NO: 10 - protein, 14 aa, synthetic construct
  REGION 1..14: note = Partial sequence of C007 mass spectrometry detection results
GQAGPPGIGIPGLR

SEQ ID NO: 11 - protein, 17 aa, synthetic construct
  REGION 1..17: note = Partial sequence of C007 mass spectrometry detection results
GQAGPPGIGIPGLRGEK

SEQ ID NO: 12 - protein, 21 aa, synthetic construct
  REGION 1..21: note = Partial sequence of C007 mass spectrometry detection results
GEKGDQGIAGFPGSPGEKGEK

SEQ ID NO: 13 - protein, 15 aa, synthetic construct
  REGION 1..15: note = Partial sequence of C007 mass spectrometry detection results
GDQGIAGFPGSPGEK

SEQ ID NO: 14 - protein, 18 aa, synthetic construct
  REGION 1..18: note = Partial sequence of C007 mass spectrometry detection results
GDQGIAGFPGSPGEKGEK

SEQ ID NO: 15 - protein, 15 aa, synthetic construct
  REGION 1..15: note = Partial sequence of C007 mass spectrometry detection results
GSIGIPGMPGSPGLK

SEQ ID NO: 16 - protein, 15 aa, synthetic construct
  REGION 1..15: note = Partial sequence of C007 mass spectrometry detection results
GSIGIPGMPGSPGLK

SEQ ID NO: 17 - protein, 18 aa, synthetic construct
  REGION 1..18: note = Partial sequence of C007 mass spectrometry detection results
GSPGSVGYPGSPGLPGEK

SEQ ID NO: 18 - protein, 21 aa, synthetic construct
  REGION 1..21: note = Partial sequence of C007 mass spectrometry detection results
GSPGSVGYPGSPGLPGEKGDK

SEQ ID NO: 19 - protein, 12 aa, synthetic construct
  REGION 1..12: note = Partial sequence of C007 mass spectrometry detection results
GLPGLDGIPGVK

SEQ ID NO: 20 - protein, 30 aa, synthetic construct
  REGION 1..30: note = Partial sequence of C007 mass spectrometry detection results
GLPGLDGIPGVKGEAGLPGTPGPTGPAGQK

SEQ ID NO: 21 - protein, 18 aa, synthetic construct
  REGION 1..18: note = Partial sequence of C007 mass spectrometry detection results
GEAGLPGTPGPTGPAGQK

SEQ ID NO: 22 - protein, 23 aa, synthetic construct
  REGION 1..23: note = Partial sequence of C007 mass spectrometry detection results
GEPGSDGIPGSAGEKGEPGLPGR

SEQ ID NO: 23 - protein, 8 aa, synthetic construct
  REGION 1..8: note = Partial sequence of C007 mass spectrometry detection results
GEPGLPGR

SEQ ID NO: 24 - protein, 9 aa, synthetic construct
  REGION 1..9: note = Partial sequence of C007 mass spectrometry detection results
GFPGFPGAK

SEQ ID NO: 25 - protein, 22 aa, synthetic construct
  REGION 1..22: note = Partial sequence of C007 mass spectrometry detection results
KGSKGEVGFPGLAGSPGIPGSK

SEQ ID NO: 26 - protein, 18 aa, synthetic construct
  REGION 1..18: note = Partial sequence of C007 mass spectrometry detection results
GEVGFPGLAGSPGIPGSK

SEQ ID NO: 27 - protein, 26 aa, synthetic construct
  REGION 1..26: note = Partial sequence of C007 mass spectrometry detection results
GEQGFMGPPGPQGQPGLPGSPGHATE

SEQ ID NO: 28 - protein, 26 aa, synthetic construct
  REGION 1..26: note = Partial sequence of C007 mass spectrometry detection results
GEQGFMGPPGPQGQPGLPGSPGHATE

SEQ ID NO: 29 - protein, 15 aa, synthetic construct
  REGION 1..15: note = Partial sequence of C4P7E5 mass spectrometry detection results
GLPGTPGPTGPAGQK

SEQ ID NO: 30 - protein, 30 aa, synthetic construct
  REGION 1..30: note = Partial sequence of C4P7E5 mass spectrometry detection results
GLPGTPGPTGPAGQKGEPGSDGIPGSAGEK

SEQ ID NO: 31 - protein, 38 aa, synthetic construct
  REGION 1..38: note = Partial sequence of C4P7E5 mass spectrometry detection results
GLPGTPGPTGPAGQKGEPGSDGIPGSAGEKGEPGLPGR

SEQ ID NO: 32 - protein, 39 aa, synthetic construct
  REGION 1..39: note = Partial sequence of C4P7E5 mass spectrometry detection results
GEVGFPGLAGSPGIPGSKGEQGFMGLPGTPGPTGPAGQK

SEQ ID NO: 33 - protein, 21 aa, synthetic construct
  REGION 1..21: note = Partial sequence of C4P7E5 mass spectrometry detection results
GEQGFMGLPGTPGPTGPAGQK

SEQ ID NO: 34 - protein, 21 aa, synthetic construct
  REGION 1..21: note = Partial sequence of C4P7E5 mass spectrometry detection results
GEQGFMGLPGTPGPTGPAGQK

SEQ ID NO: 35 - protein, 36 aa, synthetic construct
  REGION 1..36: note = Partial sequence of C4P7E5 mass spectrometry detection results
GEQGFMGLPGTPGPTGPAGQKGEPGSDGIPGSAGEK

SEQ ID NO: 36 - protein, 23 aa, synthetic construct
  REGION 1..23: note = Partial sequence of C4P7E5 mass spectrometry detection results
GEPGSDGIPGSAGEKGEPGLPGR

SEQ ID NO: 37 - protein, 8 aa, synthetic construct
  REGION 1..8: note = Partial sequence of C4P7E5 mass spectrometry detection results
GEPGLPGR

SEQ ID NO: 38 - protein, 17 aa, synthetic construct
  REGION 1..17: note = Partial sequence of C4P7E5 mass spectrometry detection results
GEPGLPGRGFPGFPGAK

SEQ ID NO: 39 - protein, 9 aa, synthetic construct
  REGION 1..9: note = Partial sequence of C4P7E5 mass spectrometry detection results
GFPGFPGAK

SEQ ID NO: 40 - protein, 12 aa, synthetic construct
  REGION 1..12: note = Partial sequence of C4P7E5 mass spectrometry detection results
GFPGFPGAKGDK

SEQ ID NO: 41 - protein, 24 aa, synthetic construct
  REGION 1..24: note = Partial sequence of C4P7E5 mass spectrometry detection results
GDKGSKGEVGFPGLAGSPGIPGSK

SEQ ID NO: 42 - protein, 21 aa, synthetic construct
  REGION 1..21: note = Partial sequence of C4P7E5 mass spectrometry detection results
GSKGEVGFPGLAGSPGIPGSK

SEQ ID NO: 43 - protein, 18 aa, synthetic construct
  REGION 1..18: note = Partial sequence of C4P7E5 mass spectrometry detection results
GEVGFPGLAGSPGIPGSK

SEQ ID NO: 44 - protein, 24 aa, synthetic construct
  REGION 1..24: note = Partial sequence of C4P7E5 mass spectrometry detection results
GEVGFPGLAGSPGIPGSKGEQGFM

SEQ ID NO: 45 - protein, 9 aa, synthetic construct
  REGION 1..9: note = Partial sequence of C4P7C6 mass spectrometry detection results
GFPGFPGAK

SEQ ID NO: 46 - protein, 33 aa, synthetic construct
  REGION 1..33: note = Partial sequence of C4P7C6 mass spectrometry detection results
GEQGFMGPPGPQGQPGLPGSPGHAGFPGFPGAK

SEQ ID NO: 47 - protein, 33 aa, synthetic construct; identical to SEQ ID NO: 46
  REGION 1..33: note = Partial sequence of C4P7C6 mass spectrometry detection results

SEQ ID NO: 48 - protein, 24 aa, synthetic construct
  REGION 1..24: note = Partial sequence of C4P7C6 mass spectrometry detection results
GDKGSKGEVGFPGLAGSPGIPGSK

SEQ ID NO: 49 - protein, 21 aa, synthetic construct
  REGION 1..21: note = Partial sequence of C4P7C6 mass spectrometry detection results
GSKGEVGFPGLAGSPGIPGSK

SEQ ID NO: 50 - protein, 18 aa, synthetic construct
  REGION 1..18: note = Partial sequence of C4P7C6 mass spectrometry detection results
GEVGFPGLAGSPGIPGSK

SEQ ID NO: 51 - protein, 24 aa, synthetic construct
  REGION 1..24: note = Partial sequence of C4P7C6 mass spectrometry detection results
GEQGFMGPPGPQGQPGLPGSPGHA

SEQ ID NO: 52 - protein, 24 aa, synthetic construct
  REGION 1..24: note = Partial sequence of C4P7C6 mass spectrometry detection results
GEQGFMGPPGPQGQPGLPGSPGHA